European Patent Application EP 4 155 414 A1, published March 29, 2023. Title: InDel MOLECULAR MARKER OF hisD GENE OF ULTRASONICALLY-MUTAGENIZED SALMONELLA TYPHIMURIUM AND USE THEREOF. Applicant: Jiangsu University. The sequence listing filed with the application follows.

SEQUENCE LISTING (21 sequences)

SEQ ID NO: 1 - DNA, 24 bp, Artificial Sequence
  Forward primer
atggagtaaagaccatgagcttca

SEQ ID NO: 2 - DNA, 20 bp, Artificial Sequence
  Reverse primer
tgcttgctccttgagggcgt

SEQ ID NO: 3 - DNA, 1305 bp, Salmonella typhimurium
atgagcttcaataccctgattgactggaacagctgtagccctgaacagcagcgtgcgctgctgacgcgtccggcgatttccgcctctgacagtattacccggacggtcagcgatattctggataatgtaaaaacgcgcggtgacgatgccctgcgtgaatacagcgctaaatttgataaaacagaagtgacagcgctacgcgtcacccctgaagagatcgccgccgccggcgcgcgtctgagcgacgaattaaaacaggcgatgaccgctgccgtcaaaaatattgaaacgttccattccgcgcagacgctaccgcctgtagatgtggaaacccagccaggcgtgcgttgccagcaggttacgcgtcccgtctcgtctgtcggtctgtatattcccggcggctcggctccgctcttctcaacggtgctgatgctggcgacgccggcgcgcattgcgggatgccagaaggtggttctgtgctcgccgccgcccatcgctgatgaaatcctctatgcggcgcaactgtgtggcgtgcaggaaatctttaacgtcggcggcgcgcaggcgattgccgctctggccttcggcagcgagtccgtaccgaaagtggataaaatttttggccccggcaacgcctttgtaaccgaagccaaacgtcaggtcagccagcgtctcgacggcgcggctatcgatatgccagccgggccgtctgaagtactggtgatcgcagacagcggcgcaacaccggatttcgtcgcttctgacctgctctcccaggctgagcacggcccggattcccaggtgatcctgctgacgcctgatgctgacattgcccgcaaggtggcggaggcggtagaacgtcaactggcggaactgccgcgcgcggacaccgcccggcaggccctgagcgccagtcgtctgattgtgaccaaagatttagcgcagtgcgtcgccatctctaatcagtatgggccggaacacttaatcatccagacgcgcaatgcgcgcgatttggtggatgcgattaccagcgcaggctcggtatttctcggcgactggtcgccggaatccgccggtgattacgcttccggaaccaaccatgttttaccgacctatggctatactgctacctgttccagccttgggttagcggatttccagaaacggatgaccgttcaggaactgtcgaaagcgggcttttccgctctggcatcaaccattgaaacattggcggcggcagaacgtctgaccgcccataaaaatgccgtgaccctgcgcgtaaacgccctcaaggagcaagcatga

SEQ ID NO: 4 - DNA, 110 bp, Salmonella typhimurium
cctgatgctgacattgcccgcaaggtggcggaggcggtagaacgtcaactggcggaactgccgcgcgcggacaccgcccggcaggccctgagcgccagtcgtctgattgt

SEQ ID NO: 5 - DNA, 84 bp, Salmonella typhimurium
gcccgcaaggtggcggaggcggtagaacgtcaactggcggaactgccgcgcgcggacaccgccggcaggccctgagcgccagtc

SEQ ID NO: 6 - DNA, 85 bp, Salmonella typhimurium
gcccgcaaggtggcggaggcggtagaacgtcaactggcggaactgccgcgcgcggacaccgcccggcaggccctgagcgccagtc

SEQ ID NO: 7 - DNA, 127 bp, Salmonella typhimurium
gcccgcaaggtggcggaggcggtagaacgtcaactggcggaactgccgcgcgcggacaccgccggcaggacgtcaactggcggaactgccgcgcgcggacaccgccggcaggccctgagcgccagtc

SEQ ID NO: 8 - DNA, 118 bp, Salmonella typhimurium
gcccgcaaggtggcggaggcggtagaacgtcaacgcccgcaaggtggcggaggcggtagaacgtcaactggcggaactgccgcgcgcggacaccgccggcaggccctgagcgccagtc

SEQ ID NO: 9 - DNA, 112 bp, Salmonella typhimurium
gcccgcaaggtggcggaggcggtagaacgtcaactggcggaactgccgcgcgcggacaccgctggcggaactgccgcgcgcggacaccgccggcaggccctgagcgccagtc

SEQ ID NO: 10 - DNA, 109 bp, Salmonella typhimurium
gcccgcaaggtggcggaggcggtagaacgtcaactggcggaactgccgcgcgcggacactggcggaactgccgcgcgcggacaccgccggcaggccctgagcgccagtc

SEQ ID NO: 11 - DNA, 106 bp, Salmonella typhimurium
gcccgcaaggtggcggaggcggtagaacgtcaactggcggaactgccgcgcgcggacaccgccactgccgcgcgcggacaccgccggcaggccctgagcgccagtc

SEQ ID NO: 12 - DNA, 103 bp, Salmonella typhimurium
gcccgcaaggtggcggaggcggtagaacgtcaactggcggaactgccgcgaactggcggaactgccgcgcgcggacaccgccggcaggccctgagcgccagtc

SEQ ID NO: 13 - DNA, 100 bp, Salmonella typhimurium
gcccgcaaggtggcggaggcggtagaacgtcaactggcggaactgccgcgcgcggacaccgccgcgcgcggacaccgccggcaggccctgagcgccagtc

SEQ ID NO: 14 - DNA, 94 bp, Salmonella typhimurium
gcccgcaaggtggcggaggcggtagaacgtcaactggcggaaactggcggaactgccgcgcgcggacaccgccggcaggccctgagcgccagtc

SEQ ID NO: 15 - DNA, 94 bp, Salmonella typhimurium
gcccgcaaggtggcggaggcggtagaacgtcaactggcggaacctggcggaactgccgcgcgcggacaccgccggcaggccctgagcgccagtc

SEQ ID NO: 16 - DNA, 94 bp, Salmonella typhimurium
gcccgcaaggtggcggaggcggtagaacgtcaactggcggaactgccgcgcgcggacaccgccggcaggccctggcaggccctgagcgccagtc

SEQ ID NO: 17 - DNA, 91 bp, Salmonella typhimurium
gcccgcaaggtggcggaggcggtagaacgtcaaccgtcaactggcggaactgccgcgcgcggacaccgccggcaggccctgagcgccagtc

SEQ ID NO: 18 - DNA, 91 bp, Salmonella typhimurium
gcccgcaaggtggcggaggcggtagaacgtcaactggcggaacgcggaactgccgcgcgcggacaccgccggcaggccctgagcgccagtc

SEQ ID NO: 19 - DNA, 55 bp, Salmonella typhimurium
gcccgcaaggtggcggaggcggtagaacgtcaacggcaggccctgagcgccagtc

SEQ ID NO: 20 - DNA, 19 bp, Artificial Sequence
  Forward primer
gtcaggtcagccagcgtct

SEQ ID NO: 21 - DNA, 20 bp, Artificial Sequence
  Reverse primer
gtaatcgcatccaccaaatc